European Patent Application EP 4 596 718 A1, published August 6, 2025. Title: Composition for Diagnosing Pancreatic Cancer. Applicant: HuVet bio, Inc. The sequence listing filed with the application follows.

SEQUENCE LISTING (63 sequences)

SEQ ID NO: 1 - DNA, 22 bp, synthetic construct
  misc_feature 1..22: note = Primer-F(IFNL1)
  source 1..22: mol_type = other DNA
ggttcaaatctctgtcaccaca

SEQ ID NO: 2 - DNA, 20 bp, synthetic construct
  misc_feature 1..20: note = Primer-R(IFNL1)
  source 1..20: mol_type = other DNA
gaagacaggagagctgcaac

SEQ ID NO: 3 - DNA, 20 bp, synthetic construct
  misc_feature 1..20: note = Probe(IFNL1)
  source 1..20: mol_type = other DNA
tcaagaaggccagggacgcc

SEQ ID NO: 4 - DNA, 23 bp, synthetic construct
  misc_feature 1..23: note = Primer-F(IFNG)
  source 1..23: mol_type = other DNA
gcaacaaaaagaaacgagatgac

SEQ ID NO: 5 - DNA, 20 bp, synthetic construct
  misc_feature 1..20: note = Primer-R(IFNG)
  source 1..20: mol_type = other DNA
cgacagttcagccatcactt

SEQ ID NO: 6 - DNA, 27 bp, synthetic construct
  misc_feature 1..27: note = Probe(IFNG)
  source 1..27: mol_type = other DNA
tcggtaactgacttgaatgtccaacgc

SEQ ID NO: 7 - DNA, 24 bp, synthetic construct
  misc_feature 1..24: note = Primer-F(I-TAC)
  source 1..24: mol_type = other DNA
tattgtgtgctacagttgttcaag

SEQ ID NO: 8 - DNA, 23 bp, synthetic construct
  misc_feature 1..23: note = Primer-R(I-TAC)
  source 1..23: mol_type = other DNA
ggtacattatggaggctttctca

SEQ ID NO: 9 - DNA, 25 bp, synthetic construct
  misc_feature 1..25: note = Probe(I-TAC)
  source 1..25: mol_type = other DNA
tgccactttcactgcttttacccca

SEQ ID NO: 10 - DNA, 19 bp, synthetic construct
  misc_feature 1..19: note = Primer-F(TNF)
  source 1..19: mol_type = other DNA
tgcactttggagtgatcgg

SEQ ID NO: 11 - DNA, 20 bp, synthetic construct
  misc_feature 1..20: note = Primer-R(TNF)
  source 1..20: mol_type = other DNA
tcagcttgagggtttgctac

SEQ ID NO: 12 - DNA, 22 bp, synthetic construct
  misc_feature 1..22: note = Probe(TNF)
  source 1..22: mol_type = other DNA
agatgatctgactgcctgggcc

SEQ ID NO: 13 - DNA, 22 bp, synthetic construct
  misc_feature 1..22: note = Primer-F(IFNB1)
  source 1..22: mol_type = other DNA
gaaactgaagatctcctagcct

SEQ ID NO: 14 - DNA, 21 bp, synthetic construct
  misc_feature 1..21: note = Primer-R(IFNB1)
  source 1..21: mol_type = other DNA
gccatcagtcacttaaacagc

SEQ ID NO: 15 - DNA, 25 bp, synthetic construct
  misc_feature 1..25: note = Probe(IFNB1)
  source 1..25: mol_type = other DNA
tgaagcaattgtccagtcccagagg

SEQ ID NO: 16 - DNA, 18 bp, synthetic construct
  misc_feature 1..18: note = Primer-F(IFNA1)
  source 1..18: mol_type = other DNA
ggaggttgtcagagcaga

SEQ ID NO: 17 - DNA, 23 bp, synthetic construct
  misc_feature 1..23: note = Primer-R(IFNA1)
  source 1..23: mol_type = other DNA
aatgacagaattcatgaaagcgt

SEQ ID NO: 18 - DNA, 32 bp, synthetic construct
  misc_feature 1..32: note = Probe(IFNA1)
  source 1..32: mol_type = other DNA
tgagatccctctctttatcaacaaacttgcaa

SEQ ID NO: 19 - DNA, 22 bp, synthetic construct
  misc_feature 1..22: note = Primer-F(DECTIN1)
  source 1..22: mol_type = other DNA
gactctcaaagcaataccagga

SEQ ID NO: 20 - DNA, 23 bp, synthetic construct
  misc_feature 1..23: note = Primer-R(DECTIN1)
  source 1..23: mol_type = other DNA
ccacagctatcaccagtattacc

SEQ ID NO: 21 - DNA, 25 bp, synthetic construct
  misc_feature 1..25: note = Probe(DECTIN1)
  source 1..25: mol_type = other DNA
tgcagcacacgatcctttctctgaa

SEQ ID NO: 22 - DNA, 18 bp, synthetic construct
  misc_feature 1..18: note = Primer-F(CXCL8)
  source 1..18: mol_type = other DNA
tgtctggaccccaaggaa

SEQ ID NO: 23 - DNA, 24 bp, synthetic construct
  misc_feature 1..24: note = Primer-R(CXCL8)
  source 1..24: mol_type = other DNA
catcttcactgattcttggatacc

SEQ ID NO: 24 - DNA, 23 bp, synthetic construct
  misc_feature 1..23: note = Probe(CXCL8)
  source 1..23: mol_type = other DNA
acttctccacaaccctctgcacc

SEQ ID NO: 25 - DNA, 23 bp, synthetic construct
  misc_feature 1..23: note = Primer-F(FOXP3)
  source 1..23: mol_type = other DNA
ctacttcaagttccacaacatgc

SEQ ID NO: 26 - DNA, 23 bp, synthetic construct
  misc_feature 1..23: note = Primer-R(FOXP3)
  source 1..23: mol_type = other DNA
ccagtggtagatctcattgagtg

SEQ ID NO: 27 - DNA, 23 bp, synthetic construct
  misc_feature 1..23: note = Probe(FOXP3)
  source 1..23: mol_type = other DNA
cctttcacctacgccacgctcat

SEQ ID NO: 28 - DNA, 20 bp, synthetic construct
  misc_feature 1..20: note = Primer-F(VEGFA)
  source 1..20: mol_type = other DNA
gtacaagatccgcagacgtg

SEQ ID NO: 29 - DNA, 23 bp, synthetic construct
  misc_feature 1..23: note = Primer-R(VEGFA)
  source 1..23: mol_type = other DNA
ttctgtatcagtctttcctggtg

SEQ ID NO: 30 - DNA, 24 bp, synthetic construct
  misc_feature 1..24: note = Probe(VEGFA)
  source 1..24: mol_type = other DNA
tcgtttaactcaagctgcctcgcc

SEQ ID NO: 31 - DNA, 18 bp, synthetic construct
  misc_feature 1..18: note = Primer-F(CCL2)
  source 1..18: mol_type = other DNA
agcagccaccttcattcc

SEQ ID NO: 32 - DNA, 20 bp, synthetic construct
  misc_feature 1..20: note = Primer-R(CCL2)
  source 1..20: mol_type = other DNA
gcctctgcactgagatcttc

SEQ ID NO: 33 - DNA, 21 bp, synthetic construct
  misc_feature 1..21: note = Probe(CCL2)
  source 1..21: mol_type = other DNA
tcaatgccccagtcacctgct

SEQ ID NO: 34 - DNA, 21 bp, synthetic construct
  misc_feature 1..21: note = Primer-F(CCL5)
  source 1..21: mol_type = other DNA
gctgtcatcctcattgctact

SEQ ID NO: 35 - DNA, 22 bp, synthetic construct
  misc_feature 1..22: note = Primer-R(CCL5)
  source 1..22: mol_type = other DNA
tgccactggtgtagaaatactc

SEQ ID NO: 36 - DNA, 24 bp, synthetic construct
  misc_feature 1..24: note = Probe(CCL5)
  source 1..24: mol_type = other DNA
atctgcctccccatattcctcgga

SEQ ID NO: 37 - DNA, 26 bp, synthetic construct
  misc_feature 1..26: note = Primer-F(CCR5)
  source 1..26: mol_type = other DNA
gtctatatgattgatttgcacagctc

SEQ ID NO: 38 - DNA, 24 bp, synthetic construct
  misc_feature 1..24: note = Primer-R(CCR5)
  source 1..24: mol_type = other DNA
tcatagattggacttgacacttga

SEQ ID NO: 39 - DNA, 25 bp, synthetic construct
  misc_feature 1..25: note = Probe(CCR5)
  source 1..25: mol_type = other DNA
cgttcccctacaagaaactctcccc

SEQ ID NO: 40 - DNA, 19 bp, synthetic construct
  misc_feature 1..19: note = Primer-F(CXCR4)
  source 1..19: mol_type = other DNA
agcaggtagcaaagtgacg

SEQ ID NO: 41 - DNA, 23 bp, synthetic construct
  misc_feature 1..23: note = Primer-R(CXCR4)
  source 1..23: mol_type = other DNA
cctcggtgtagttatctgaagtg

SEQ ID NO: 42 - DNA, 21 bp, synthetic construct
  misc_feature 1..21: note = Probe(CXCR4)
  source 1..21: mol_type = other DNA
agatgcggtggctactggagc

SEQ ID NO: 43 - DNA, 20 bp, synthetic construct
  misc_feature 1..20: note = Primer-F(ARG1)
  source 1..20: mol_type = other DNA
actccactgacaaccacaag

SEQ ID NO: 44 - DNA, 21 bp, synthetic construct
  misc_feature 1..21: note = Primer-R(ARG1)
  source 1..21: mol_type = other DNA
tggcagatatacagggagtca

SEQ ID NO: 45 - DNA, 29 bp, synthetic construct
  misc_feature 1..29: note = Probe(ARG1)
  source 1..29: mol_type = other DNA
ccttcaggaggaaagatacaggttgtcca

SEQ ID NO: 46 - DNA, 19 bp, synthetic construct
  misc_feature 1..19: note = Primer-F(CXCR2)
  source 1..19: mol_type = other DNA
tctgactaccacccaacct

SEQ ID NO: 47 - DNA, 20 bp, synthetic construct
  misc_feature 1..20: note = Primer-R(CXCR2)
  source 1..20: mol_type = other DNA
ctgggcttttcacctgtagg

SEQ ID NO: 48 - DNA, 26 bp, synthetic construct
  misc_feature 1..26: note = Probe(CXCR2)
  source 1..26: mol_type = other DNA
ccactccaataacagcaggtcacagc

SEQ ID NO: 49 - DNA, 25 bp, synthetic construct
  misc_feature 1..25: note = Primer-F(FATP2)
  source 1..25: mol_type = other DNA
ctgtcattcagtatatcggtgaact

SEQ ID NO: 50 - DNA, 21 bp, synthetic construct
  misc_feature 1..21: note = Primer-R(FATP2)
  source 1..21: mol_type = other DNA
atctcctcgtaagccatttcc

SEQ ID NO: 51 - DNA, 27 bp, synthetic construct
  misc_feature 1..27: note = Probe(FATP2)
  source 1..27: mol_type = other DNA
tgcaactcaccacagaaaccaaatgac

SEQ ID NO: 52 - DNA, 23 bp, synthetic construct
  misc_feature 1..23: note = Primer-F(PTGS2)
  source 1..23: mol_type = other DNA
gcactacatacttacccacttca

SEQ ID NO: 53 - DNA, 23 bp, synthetic construct
  misc_feature 1..23: note = Primer-R(PTGS2)
  source 1..23: mol_type = other DNA
gccatagtcagcattgtaagttg

SEQ ID NO: 54 - DNA, 30 bp, synthetic construct
  misc_feature 1..30: note = Probe(PTGS2)
  source 1..30: mol_type = other DNA
acatccagatcacatttgattgacagtcca

SEQ ID NO: 55 - DNA, 23 bp, synthetic construct
  misc_feature 1..23: note = Primer-F(PTGES2)
  source 1..23: mol_type = other DNA
gcaacaactaaatgactcctctg

SEQ ID NO: 56 - DNA, 23 bp, synthetic construct
  misc_feature 1..23: note = Primer-R(PTGES2)
  source 1..23: mol_type = other DNA
ctgggtagtaggtgatgatctct

SEQ ID NO: 57 - DNA, 23 bp, synthetic construct
  misc_feature 1..23: note = Probe(PTGES2)
  source 1..23: mol_type = other DNA
cccgacaccaggtaggtcttgag

SEQ ID NO: 58 - DNA, 17 bp, synthetic construct
  misc_feature 1..17: note = Primer-F(PTGES)
  source 1..17: mol_type = other DNA
gtggaacgctgcctcag

SEQ ID NO: 59 - DNA, 21 bp, synthetic construct
  misc_feature 1..21: note = Primer-R(PTGES)
  source 1..21: mol_type = other DNA
ccagaaaggagtagacgaagc

SEQ ID NO: 60 - DNA, 25 bp, synthetic construct
  misc_feature 1..25: note = Probe(PTGES)
  source 1..25: mol_type = other DNA
aggaaggggtagatggtctccatgt

SEQ ID NO: 61 - DNA, 19 bp, synthetic construct
  misc_feature 1..19: note = Primer-F(GAPDH)
  source 1..19: mol_type = other DNA
acatcgctcagacaccatg

SEQ ID NO: 62 - DNA, 22 bp, synthetic construct
  misc_feature 1..22: note = Primer-R(GAPDH)
  source 1..22: mol_type = other DNA
tgtagttgaggtcaatgaaggg

SEQ ID NO: 63 - DNA, 25 bp, synthetic construct
  misc_feature 1..25: note = Probe(GAPDH)
  source 1..25: mol_type = other DNA
aaggtcggagtcaacggatttggtc